European Patent Application EP 4 458 985 A1, published November 6, 2024. Title: 多种靶核酸检测的方法. Applicant: 迈克生物股份有限公司. The sequence listing filed with the application follows.

SEQUENCE LISTING (14 sequences)

SEQ ID NO: 1 - DNA, 59 bp, synthetic construct
  source 1..59: mol_type = other DNA
tcgaccacgtgacagtctcctcgctgacactcactgctgatcaggctccctgtgtcgca

SEQ ID NO: 2 - DNA, 39 bp, synthetic construct
  source 1..39: mol_type = other DNA
gtcacgtggtcgatttagcaaattggacttcccgtaacg

SEQ ID NO: 3 - DNA, 49 bp, synthetic construct
  source 1..49: mol_type = other DNA
ttttttctcctcgctgacactaaaccttctagagaatgcgtgggaatct

SEQ ID NO: 4 - DNA, 37 bp, synthetic construct
  source 1..37: mol_type = other DNA
gtcacgtggtcgatttaaactgacactgggctctgca

SEQ ID NO: 5 - DNA, 35 bp, synthetic construct
  source 1..35: mol_type = other DNA
cactgctgataaagtcatttgccgtgccatacact

SEQ ID NO: 6 - DNA, 35 bp, synthetic construct
  source 1..35: mol_type = other DNA
gtcacgtggtcgatttattggcgaggcacgtatga

SEQ ID NO: 7 - DNA, 37 bp, synthetic construct
  source 1..37: mol_type = other DNA
ctgtgtcgcaaaacaccgtcgagccagaaactgtcta

SEQ ID NO: 8 - DNA, 59 bp, synthetic construct
  source 1..59: mol_type = other DNA
ctgctacctcagctctgagtcaacctgacctccaatcttctgactagcgtgtgatcgtc

SEQ ID NO: 9 - DNA, 39 bp, synthetic construct
  source 1..39: mol_type = other DNA
gctgaggtagcagtttagcaaattggacttcccgtaacg

SEQ ID NO: 10 - DNA, 49 bp, synthetic construct
  source 1..49: mol_type = other DNA
ttttttgagtcaacctgacctaaaccttctagagaatgcgtgggaatct

SEQ ID NO: 11 - DNA, 35 bp, synthetic construct
  source 1..35: mol_type = other DNA
gctgaggtagcagtttattggcgaggcacgtatga

SEQ ID NO: 12 - DNA, 38 bp, synthetic construct
  source 1..38: mol_type = other DNA
ccaatcttctgaaacaccgtcgagccagaaactgtcta

SEQ ID NO: 13 - DNA, 40 bp, synthetic construct
  source 1..40: mol_type = other DNA
gctgaggtagcagttttagtagtttggctgcctgaaagga

SEQ ID NO: 14 - DNA, 35 bp, synthetic construct
  source 1..35: mol_type = other DNA
gtgatcgtcaaagtcacccaaattacctagaccgt